European Patent Application EP 4 155 321 A1, published March 29, 2023. Title: ANTI-DDR2 ANTIBODIES AND USES THEREOF. Applicant: CHUGAI SEIYAKU KABUSHIKI KAISHA. The sequence listing filed with the application follows.

SEQUENCE LISTING (102 sequences)

SEQ ID NO: 1 - protein, 124 aa, Artificial Sequence
  an artificially synthesized sequence
QSVEESGGRLVTPGTPLTLTCTVSGFSLSTSAMSWVRQAPGKGLEWIGMITYGGSGSTWYASWANGRFTISKTSTTVTLKMTSPTTEDTASYFCARVYGTIGSNFYSIYSFNLWGQGTLVTVSS

SEQ ID NO: 2 - protein, 5 aa, Artificial Sequence
  an artificially synthesized sequence
TSAMS

SEQ ID NO: 3 - protein, 18 aa, Artificial Sequence
  an artificially synthesized sequence
MITYGGSGSTWYASWANG

SEQ ID NO: 4 - protein, 17 aa, Artificial Sequence
  an artificially synthesized sequence
VYGTIGSNFYSIYSFNL

SEQ ID NO: 5 - protein, 111 aa, Artificial Sequence
  an artificially synthesized sequence
AAVLTQTPSPVSAAVGGTVSISCQSSKSVYNSNYLSWYQQKPGQPPKLLIYYTSALASGVSSRFKGSGSGTRFTLTISDVQCDDAATYYCAGGYSSSSDNGFGGGTKVEIK

SEQ ID NO: 6 - protein, 13 aa, Artificial Sequence
  an artificially synthesized sequence
QSSKSVYNSNYLS

SEQ ID NO: 7 - protein, 7 aa, Artificial Sequence
  an artificially synthesized sequence
YTSALAS

SEQ ID NO: 8 - protein, 11 aa, Artificial Sequence
  an artificially synthesized sequence
AGGYSSSSDNG

SEQ ID NO: 9 - protein, 116 aa, Artificial Sequence
  an artificially synthesized sequence
QSVEESGGRLITPGTPLTLTCTASGFSLSIYYMIWVRQAPGKGLEWIGYIWSGSTTDYASWAKGRFTISKTSTTVDLKITSPTTEDTATYFCARVYAGYGYGSDLWGQGTLVTVSS

SEQ ID NO: 10 - protein, 5 aa, Artificial Sequence
  an artificially synthesized sequence
IYYMI

SEQ ID NO: 11 - protein, 16 aa, Artificial Sequence
  an artificially synthesized sequence
YIWSGSTTDYASWAKG

SEQ ID NO: 12 - protein, 11 aa, Artificial Sequence
  an artificially synthesized sequence
VYAGYGYGSDL

SEQ ID NO: 13 - protein, 112 aa, Artificial Sequence
  an artificially synthesized sequence
AAVLTQTPSPVSAAVGGTVSISCQSSQSVYNNNWLAWYQQKPGQPPKLLIYSASTLASGVPSRFKGSGSGTQFTLTISDVQCDDAATYYCAGGYSTNSDKNAFGGGTKVEIK

SEQ ID NO: 14 - protein, 13 aa, Artificial Sequence
  an artificially synthesized sequence
QSSQSVYNNNWLA

SEQ ID NO: 15 - protein, 7 aa, Artificial Sequence
  an artificially synthesized sequence
SASTLAS

SEQ ID NO: 16 - protein, 12 aa, Artificial Sequence
  an artificially synthesized sequence
AGGYSTNSDKNA

SEQ ID NO: 17 - protein, 112 aa, Artificial Sequence
  an artificially synthesized sequence
QSVEESGGRLVTPGTALTLTCTASGFSLSSYDMSWVRQAPGEGLEWIGTIFTEGSTSCASWVKGRFTISRTSTTVDLKITSPTTEDTATYFCVRGTTSNRLWGQGTLVTVSS

SEQ ID NO: 18 - protein, 5 aa, Artificial Sequence
  an artificially synthesized sequence
SYDMS

SEQ ID NO: 19 - protein, 16 aa, Artificial Sequence
  an artificially synthesized sequence
TIFTEGSTSCASWVKG

SEQ ID NO: 20 - protein, 7 aa, Artificial Sequence
  an artificially synthesized sequence
GTTSNRL

SEQ ID NO: 21 - protein, 112 aa, Artificial Sequence
  an artificially synthesized sequence
DVVMTQTPASVEAVVGATVTIRCQASESITNYLSWYQQKPGQPPKVLIYYASTLESGVPSRFKGSGSGTQFTLTISDLECADAATYYCQSNYFSSSYSYGNTFGGGTKVEIK

SEQ ID NO: 22 - protein, 11 aa, Artificial Sequence
  an artificially synthesized sequence
QASESITNYLS

SEQ ID NO: 23 - protein, 7 aa, Artificial Sequence
  an artificially synthesized sequence
YASTLES

SEQ ID NO: 24 - protein, 14 aa, Artificial Sequence
  an artificially synthesized sequence
QSNYFSSSYSYGNT

SEQ ID NO: 25 - protein, 121 aa, Artificial Sequence
  an artificially synthesized sequence
QSVEESGGRLVTPGTPLTLTCTVSGFSLSSYSMGWVRQAPGKGLEYIGVINTSDSAYYASWAKGRFTISRTSTTVDLKMTSLTTEDTATYFCARAIGYYGSGWGACYFNLWGQGTLVTVSS

SEQ ID NO: 26 - protein, 5 aa, Artificial Sequence
  an artificially synthesized sequence
SYSMG

SEQ ID NO: 27 - protein, 16 aa, Artificial Sequence
  an artificially synthesized sequence
VINTSDSAYYASWAKG

SEQ ID NO: 28 - protein, 16 aa, Artificial Sequence
  an artificially synthesized sequence
AIGYYGSGWGACYFNL

SEQ ID NO: 29 - protein, 112 aa, Artificial Sequence
  an artificially synthesized sequence
AIKMTQTPSSVSAAVGGTVTVNCQASEDIKSYLAWYQQKPGQPPKLLIYSASTLASGVSSRFKGSGSGTQFTLTISDLECADAATYYCQSYYGTSTTGEYNAFGGGTKVEIK

SEQ ID NO: 30 - protein, 11 aa, Artificial Sequence
  an artificially synthesized sequence
QASEDIKSYLA

SEQ ID NO: 31 - protein, 7 aa, Artificial Sequence
  an artificially synthesized sequence
SASTLAS

SEQ ID NO: 32 - protein, 14 aa, Artificial Sequence
  an artificially synthesized sequence
QSYYGTSTTGEYNA

SEQ ID NO: 33 - protein, 115 aa, Artificial Sequence
  an artificially synthesized sequence
QSLEESGGRLVTPGTPLTLTCTASGFSLSNYYMQWVRQAPGKGLEWIGIVYPGSSAYYANWAKGRFTISKTSTTVDLKMTSLTTEDTATYFCAGSSNSVYSFNLWGQGTLVTVSS

SEQ ID NO: 34 - protein, 5 aa, Artificial Sequence
  an artificially synthesized sequence
NYYMQ

SEQ ID NO: 35 - protein, 16 aa, Artificial Sequence
  an artificially synthesized sequence
IVYPGSSAYYANWAKG

SEQ ID NO: 36 - protein, 10 aa, Artificial Sequence
  an artificially synthesized sequence
SSNSVYSFNL

SEQ ID NO: 37 - protein, 110 aa, Artificial Sequence
  an artificially synthesized sequence
AYDMTQTPSSVSAAVGGTVTIKCQASESIYRSLAWYQQKPGQPPKLLIYSASTLTSGVSSRFKGSGSGTEFTLTISDLECADAGTYYCQQGGSFSNIVNTFGGGTKVEIK

SEQ ID NO: 38 - protein, 11 aa, Artificial Sequence
  an artificially synthesized sequence
QASESIYRSLA

SEQ ID NO: 39 - protein, 7 aa, Artificial Sequence
  an artificially synthesized sequence
SASTLTS

SEQ ID NO: 40 - protein, 12 aa, Artificial Sequence
  an artificially synthesized sequence
QQGGSFSNIVNT

SEQ ID NO: 41 - protein, 113 aa, Artificial Sequence
  an artificially synthesized sequence
QSVEESGGRLVTPGTPLTLTCTVSGFSLSSYSVAWVRQAPGKGLEWIGYISYSGSTYYASWVNGRFTISKTSTTVDLKMTSLTASDTATYFCARDPGYSRDLWGQGTLVTVSS

SEQ ID NO: 42 - protein, 5 aa, Artificial Sequence
  an artificially synthesized sequence
SYSVA

SEQ ID NO: 43 - protein, 16 aa, Artificial Sequence
  an artificially synthesized sequence
YISYSGSTYYASWVNG

SEQ ID NO: 44 - protein, 8 aa, Artificial Sequence
  an artificially synthesized sequence
DPGYSRDL

SEQ ID NO: 45 - protein, 109 aa, Artificial Sequence
  an artificially synthesized sequence
DVVMTQTPSSVSEPVGGTVTIKCQASQSIGSYLSWYQQKPGQPPKLLIYRASTLASGVSSRFKGSGSGTEFTLTINGLECADAAIYYCQSSYVGVSHGSFGGGTKVEIK

SEQ ID NO: 46 - protein, 11 aa, Artificial Sequence
  an artificially synthesized sequence
QASQSIGSYLS

SEQ ID NO: 47 - protein, 7 aa, Artificial Sequence
  an artificially synthesized sequence
RASTLAS

SEQ ID NO: 48 - protein, 11 aa, Artificial Sequence
  an artificially synthesized sequence
QSSYVGVSHGS

SEQ ID NO: 49 - protein, 115 aa, Artificial Sequence
  an artificially synthesized sequence
QSLEESGGRLVTPGGSLTLTCTASGFSLSAYYMQWVRQAPGKGLEWIGWINTGGSAYYPSWARGRFTISKTSTTVDLKITSPTTEDTATYFCARSDASVHQFNLWGQGTLVTVSS

SEQ ID NO: 50 - protein, 5 aa, Artificial Sequence
  an artificially synthesized sequence
AYYMQ

SEQ ID NO: 51 - protein, 16 aa, Artificial Sequence
  an artificially synthesized sequence
WINTGGSAYYPSWARG

SEQ ID NO: 52 - protein, 10 aa, Artificial Sequence
  an artificially synthesized sequence
SDASVHQFNL

SEQ ID NO: 53 - protein, 111 aa, Artificial Sequence
  an artificially synthesized sequence
DVVMTQTPASVEAAVGGTVTIKCQASESIGNALAWYQQRPGQPPKLLIYYASTLESGVPSRFKGSGSGTEFTLTISDLECADAATYYCQCTYGSGSSRGNAFGGGTKVEIK

SEQ ID NO: 54 - protein, 11 aa, Artificial Sequence
  an artificially synthesized sequence
QASESIGNALA

SEQ ID NO: 55 - protein, 7 aa, Artificial Sequence
  an artificially synthesized sequence
YASTLES

SEQ ID NO: 56 - protein, 13 aa, Artificial Sequence
  an artificially synthesized sequence
QCTYGSGSSRGNA

SEQ ID NO: 57 - protein, 114 aa, Artificial Sequence
  an artificially synthesized sequence
QSVEESGGRLVTPGTPLTLTCAVSGFSLNSHVMGWVRQAPGRGLECIGIIAVSGDIYYANWAKGRFTISKTSTTVDLRITSPTTEDTATYFCGSPTVINNNNLWGQGTLVTVSS

SEQ ID NO: 58 - protein, 5 aa, Artificial Sequence
  an artificially synthesized sequence
SHVMG

SEQ ID NO: 59 - protein, 16 aa, Artificial Sequence
  an artificially synthesized sequence
IIAVSGDIYYANWAKG

SEQ ID NO: 60 - protein, 9 aa, Artificial Sequence
  an artificially synthesized sequence
PTVINNNNL

SEQ ID NO: 61 - protein, 113 aa, Artificial Sequence
  an artificially synthesized sequence
AQVLTQTASPVSAAVGGTVTINCQSSQNVYGNNYLSWFQQKPGQPPKLLIYSTSTLASGVSSRFKGSGSGTQFTLTISDLECADAATYYCLGGYDCNIVDCRAFGGGTKVEIK

SEQ ID NO: 62 - protein, 13 aa, Artificial Sequence
  an artificially synthesized sequence
QSSQNVYGNNYLS

SEQ ID NO: 63 - protein, 7 aa, Artificial Sequence
  an artificially synthesized sequence
STSTLAS

SEQ ID NO: 64 - protein, 13 aa, Artificial Sequence
  an artificially synthesized sequence
LGGYDCNIVDCRA

SEQ ID NO: 65 - protein, 116 aa, Artificial Sequence
  an artificially synthesized sequence
QSVEESGGRLVTPGTPLTLTCTVSGFSLNRYTGIWVRQAPGKGLEWIGIISSDDRTWYASWAKGRFTISKTSTTVDLKITSPTIEDTATYFCARDVGGDSWFWGLWGQGTLVTVSS

SEQ ID NO: 66 - protein, 5 aa, Artificial Sequence
  an artificially synthesized sequence
RYTGI

SEQ ID NO: 67 - protein, 16 aa, Artificial Sequence
  an artificially synthesized sequence
IISSDDRTWYASWAKG

SEQ ID NO: 68 - protein, 11 aa, Artificial Sequence
  an artificially synthesized sequence
DVGGDSWFWGL

SEQ ID NO: 69 - protein, 113 aa, Artificial Sequence
  an artificially synthesized sequence
DIVMTQTPASVEAAVGGTVTIKCQASQSISSWLAWYQQKPGQPPKLLIYYASTLASGVPSRFSGSGSGTEFTLTISDLECADAATYYCQSNYYSSSNSNYGHAFGGGTKVEIK

SEQ ID NO: 70 - protein, 11 aa, Artificial Sequence
  an artificially synthesized sequence
QASQSISSWLA

SEQ ID NO: 71 - protein, 7 aa, Artificial Sequence
  an artificially synthesized sequence
YASTLAS

SEQ ID NO: 72 - protein, 15 aa, Artificial Sequence
  an artificially synthesized sequence
QSNYYSSSNSNYGHA

SEQ ID NO: 73 - protein, 328 aa, Artificial Sequence
  an artificially synthesized sequence
ASTKGPSVFPLAPSSKSTSGGTAALGCLVKDYFPEPVTVSWNSGALTSGVHTFPAVLQSSGLYSLSSVVTVPSSSLGTQTYICNVNHKPSNTKVDKRVEPKSCDKTHTCPPCPAPELRRGPSVFLFPPKPKDTLMISRTPEVTCVVVDVSHEDPEVKFNWYVDGVEVHNAKTKPREEQYNSTYRVVSVLTVLHQDWLNGKEYKCKVSNKALPAPIEKTISKAKGQPREPQVYTLPPSREEMTKNQVSLTCLVKGFYPSDIAVEWESNGQPENNYKTTPPVLDSDGSFFLYSKLTVDKSRWQQGNVFSCSVMHEALHNHYTQKSLSLSP

SEQ ID NO: 74 - protein, 107 aa, Artificial Sequence
  an artificially synthesized sequence
RTVAAPSVFIFPPSDEQLKSGTASVVCLLNNFYPREAKVQWKVDNALQSGNSQESVTEQDSKDCTYSLSSTLTLSKADYEKHKVYACEVTHQGLSSPVTKSFNRGEC

SEQ ID NO: 75 - protein, 324 aa, Artificial Sequence
  an artificially synthesized sequence
AKTTPPSVYPLAPGSAAQTNSMVTLGCLVKGYFPEPVTVTWNSGSLSSGVHTFPAVLQSDLYTLSSSVTVPSSTWPSETVTCNVAHPASSTKVDKKIVPRDCGCKPCICTVKEVSKVFIFPPKPKDVLTITLTPKVTCVVVDISKDDPEVQFSWFVDDVEVHTAQTQPREEQFNSTFRSVSELPIMHQDWLNGKEFKCRVNSAAFPAPIEKTISKTKGRPKAPQVYTIPPPKEQMAKDKVSLTCMITDFFPEDITVEWQWNGQPAENYKNTQPIMDTDGSYFVYSKLNVQKSNWEAGNTFTCSVLHEGLHNHHTEKSLSHSPGK

SEQ ID NO: 76 - protein, 107 aa, Artificial Sequence
  an artificially synthesized sequence
RADAAPTVSIFPPSSEQLTSGGASVVCFLNNFYPKDINVKWKIDGSERQNGVLNSWTDQDSKDSTYSMSSTLTLTKDEYERHNSYTCEATHKTSTSPIVKSFNRNEC

SEQ ID NO: 77 - protein, 854 aa, Mus musculus
MIPIPRMPLVLLLLLLILGSAKAQVNPAICRYPLGMSGGHIPDEDITASSQWSESTAAKYGRLDSEEGDGAWCPEIPVQPDDLKEFLQIDLRTLHFITLVGTQGRHAGGHGIEFAPMYKINYSRDGSRWISWRNRHGKQVLDGNSNPYDVFLKDLEPPIVARFVRLIPVTDHSMNVCMRVELYGCVWLDGLVSYNAPAGQQFVLPGGSIIYLNDSVYDGAVGYSMTEGLGQLTDGVSGLDDFTQTHEYHVWPGYDYVGWRNESATNGFIEIMFEFDRIRNFTTMKVHCNNMFAKGVKIFKEVQCYFRSEASEWEPTAVYFPLVLDDVNPSARFVTVPLHHRMASAIKCQYHFADTWMMFSEITFQSDAAMYNNSGALPTSPMAPTTYDPMLKVDDSNTRILIGCLVAIIFILLAIIVIILWRQFWQKMLEKASRRMLDDEMTVSLSLPSESSMFNNNRSSSPSEQESNSTYDRIFPLRPDYQEPSRLIRKLPEFAPGEEESGCSGVVKPAQPNGPEGVPHYAEADIVNLQGVTGGNTYCVPAVTMDLLSGKDVAVEEFPRKLLAFKEKLGEGQFGEVHLCEVEGMEKFKDKDFALDVSANQPVLVAVKMLRADANKNARNDFLKEIKIMSRLKDPNIIRLLAVCITEDPLCMITEYMENGDLNQFLSRHEPLSSCSSDATVSYANLKFMATQIASGMKYLSSLNFVHRDLATRNCLVGKNYTIKIADFGMSRNLYSGDYYRIQGRAVLPIRWMSWESILLGKFTTASDVWAFGVTLWETFTFCQEQPYSQLSDEQVIENTGEFFRDQGRQIYLPQPALCPDSVYKLMLSCWRRETKHRPSFQEIHLLLLQQGAE

SEQ ID NO: 78 - protein, 855 aa, Homo sapiens
MILIPRMLLVLFLLLPILSSAKAQVNPAICRYPLGMSGGQIPDEDITASSQWSESTAAKYGRLDSEEGDGAWCPEIPVEPDDLKEFLQIDLHTLHFITLVGTQGRHAGGHGIEFAPMYKINYSRDGTRWISWRNRHGKQVLDGNSNPYDIFLKDLEPPIVARFVRFIPVTDHSMNVCMRVELYGCVWLDGLVSYNAPAGQQFVLPGGSIIYLNDSVYDGAVGYSMTEGLGQLTDGVSGLDDFTQTHEYHVWPGYDYVGWRNESATNGYIEIMFEFDRIRNFTTMKVHCNNMFAKGVKIFKEVQCYFRSEASEWEPNAISFPLVLDDVNPSARFVTVPLHHRMASAIKCQYHFADTWMMFSEITFQSDAAMYNNSEALPTSPMAPTTYDPMLKVDDSNTRILIGCLVAIIFILLAIIVIILWRQFWQKMLEKASRRMLDDEMTVSLSLPSDSSMFNNNRSSSPSEQGSNSTYDRIFPLRPDYQEPSRLIRKLPEFAPGEEESGCSGVVKPVQPSGPEGVPHYAEADIVNLQGVTGGNTYSVPAVTMDLLSGKDVAVEEFPRKLLTFKEKLGEGQFGEVHLCEVEGMEKFKDKDFALDVSANQPVLVAVKMLRADANKNARNDFLKEIKIMSRLKDPNIIHLLAVCITDDPLCMITEYMENGDLNQFLSRHEPPNSSSSDVRTVSYTNLKFMATQIASGMKYLSSLNFVHRDLATRNCLVGKNYTIKIADFGMSRNLYSGDYYRIQGRAVLPIRWMSWESILLGKFTTASDVWAFGVTLWETFTFCQEQPYSQLSDEQVIENTGEFFRDQGRQTYLPQPAICPDSVYKLMLSCWRRDTKNRPSFQEIHLLLLQQGDE

SEQ ID NO: 79 - protein, 911 aa, Mus musculus
MGTGTLSSLLLLLLLVTIGDADMKGHFDPAKCRYALGMQDRTIPDSDISVSSSWSDSTAARHSRLESSDGDGAWCPAGPVFPKEEEYLQVDLRRLHLVALVGTQGRHAGGLGKEFSRSYRLRYSRDGRRWMDWKDRWGQEVISGNEDPGGVVLKDLGPPMVARLVRFYPRADRVMSVCLRVELYGCLWRDGLLSYTAPVGQTMQLSEVMVHLNDSTYDGYTAGGLQYGGLGQLADGVVGLDDFRQSQELRVWPGYDYVGWSNQSFPTGYVEMEFEFDRLRTFQTMQVHCNNMHTLGARLPGGVECRFKRGPAMAWEGEPVRHALGGSLGDPRARAISVPLGGHVGRFLQCRFLFAGPWLLFSEISFISDVVNDSSDTFPPAPWWPPGPPPTNFSSLELEPRGQQPVAKAEGSPTAILIGCLVAIILLLLLIIALMLWRLHWRRLLSKAERRVLEEELTVHLSVPGDTILINNRPGPREPPPYQEPRPRGTPPHSAPCVPNGSALLLSNPAYRLLLATYARPPRGPGPPTPAWAKPTNTQACSGDYMEPEKPGAPLLPPPPQNSVPHYAEADIVTLQGVTGGNTYAVPALPPGAVGDGPPRVDFPRSRLRFKEKLGEGQFGEVHLCEVEDPQDLVSSDFPISVHKGHPLLVAVKILRPDATKNARNDFLKEVKIMSRLKDPNIIRLLGVCVQDDPLCMITDYMENGDLNQFLSARQLENKATQGLSGDTESDQGPTISYPMLLHVGAQIASGMRYLATLNFVHRDLATRNCLVGENFTIKIADFGMSRNLYAGDYYRVQGRAVLPIRWMAWECILMGKFTTASDVWAFGVTLWEVLMLCRSQPFGQLTDEQVIENAGEFFRDQGRQVYLSRPPACPQTLYELMLRCWSREPEQRPPFAQLHRFLADDALNTV

SEQ ID NO: 80 - protein, 913 aa, Homo sapiens
MGPEALSSLLLLLLVASGDADMKGHFDPAKCRYALGMQDRTIPDSDISASSSWSDSTAARHSRLESSDGDGAWCPAGSVFPKEEEYLQVDLQRLHLVALVGTQGRHAGGLGKEFSRSYRLRYSRDGRRWMGWKDRWGQEVISGNEDPEGVVLKDLGPPMVARLVRFYPRADRVMSVCLRVELYGCLWRDGLLSYTAPVGQTMYLSEAVYLNDSTYDGHTVGGLQYGGLGQLADGVVGLDDFRKSQELRVWPGYDYVGWSNHSFSSGYVEMEFEFDRLRAFQAMQVHCNNMHTLGARLPGGVECRFRRGPAMAWEGEPMRHNLGGNLGDPRARAVSVPLGGRVARFLQCRFLFAGPWLLFSEISFISDVVNNSSPALGGTFPPAPWWPPGPPPTNFSSLELEPRGQQPVAKAEGSPTAILIGCLVAIILLLLLIIALMLWRLHWRRLLSKAERRVLEEELTVHLSVPGDTILINNRPGPREPPPYQEPRPRGNPPHSAPCVPNGSALLLSNPAYRLLLATYARPPRGPGPPTPAWAKPTNTQAYSGDYMEPEKPGAPLLPPPPQNSVPHYAEADIVTLQGVTGGNTYAVPALPPGAVGDGPPRVDFPRSRLRFKEKLGEGQFGEVHLCEVDSPQDLVSLDFPLNVRKGHPLLVAVKILRPDATKNARNDFLKEVKIMSRLKDPNIIRLLGVCVQDDPLCMITDYMENGDLNQFLSAHQLEDKAAEGAPGDGQAAQGPTISYPMLLHVAAQIASGMRYLATLNFVHRDLATRNCLVGENFTIKIADFGMSRNLYAGDYYRVQGRAVLPIRWMAWECILMGKFTTASDVWAFGVTLWEVLMLCRAQPFGQLTDEQVIENAGEFFRDQGRQVYLSRPPACPQGLYELMLRCWSRESEQRPPFSQLHRFLAEDALNTV

SEQ ID NO: 81 - protein, 876 aa, Homo sapiens
MGPEALSSLLLLLLVASGDADMKGHFDPAKCRYALGMQDRTIPDSDISASSSWSDSTAARHSRLESSDGDGAWCPAGSVFPKEEEYLQVDLQRLHLVALVGTQGRHAGGLGKEFSRSYRLRYSRDGRRWMGWKDRWGQEVISGNEDPEGVVLKDLGPPMVARLVRFYPRADRVMSVCLRVELYGCLWRDGLLSYTAPVGQTMYLSEAVYLNDSTYDGHTVGGLQYGGLGQLADGVVGLDDFRKSQELRVWPGYDYVGWSNHSFSSGYVEMEFEFDRLRAFQAMQVHCNNMHTLGARLPGGVECRFRRGPAMAWEGEPMRHNLGGNLGDPRARAVSVPLGGRVARFLQCRFLFAGPWLLFSEISFISDVVNNSSPALGGTFPPAPWWPPGPPPTNFSSLELEPRGQQPVAKAEGSPTAILIGCLVAIILLLLLIIALMLWRLHWRRLLSKAERRVLEEELTVHLSVPGDTILINNRPGPREPPPYQEPRPRGNPPHSAPCVPNGSAYSGDYMEPEKPGAPLLPPPPQNSVPHYAEADIVTLQGVTGGNTYAVPALPPGAVGDGPPRVDFPRSRLRFKEKLGEGQFGEVHLCEVDSPQDLVSLDFPLNVRKGHPLLVAVKILRPDATKNARNDFLKEVKIMSRLKDPNIIRLLGVCVQDDPLCMITDYMENGDLNQFLSAHQLEDKAAEGAPGDGQAAQGPTISYPMLLHVAAQIASGMRYLATLNFVHRDLATRNCLVGENFTIKIADFGMSRNLYAGDYYRVQGRAVLPIRWMAWECILMGKFTTASDVWAFGVTLWEVLMLCRAQPFGQLTDEQVIENAGEFFRDQGRQVYLSRPPACPQGLYELMLRCWSRESEQRPPFSQLHRFLAEDALNTV

SEQ ID NO: 82 - protein, 919 aa, Homo sapiens
MGPEALSSLLLLLLVASGDADMKGHFDPAKCRYALGMQDRTIPDSDISASSSWSDSTAARHSRLESSDGDGAWCPAGSVFPKEEEYLQVDLQRLHLVALVGTQGRHAGGLGKEFSRSYRLRYSRDGRRWMGWKDRWGQEVISGNEDPEGVVLKDLGPPMVARLVRFYPRADRVMSVCLRVELYGCLWRDGLLSYTAPVGQTMYLSEAVYLNDSTYDGHTVGGLQYGGLGQLADGVVGLDDFRKSQELRVWPGYDYVGWSNHSFSSGYVEMEFEFDRLRAFQAMQVHCNNMHTLGARLPGGVECRFRRGPAMAWEGEPMRHNLGGNLGDPRARAVSVPLGGRVARFLQCRFLFAGPWLLFSEISFISDVVNNSSPALGGTFPPAPWWPPGPPPTNFSSLELEPRGQQPVAKAEGSPTAILIGCLVAIILLLLLIIALMLWRLHWRRLLSKAERRVLEEELTVHLSVPGDTILINNRPGPREPPPYQEPRPRGNPPHSAPCVPNGSALLLSNPAYRLLLATYARPPRGPGPPTPAWAKPTNTQAYSGDYMEPEKPGAPLLPPPPQNSVPHYAEADIVTLQGVTGGNTYAVPALPPGAVGDGPPRVDFPRSRLRFKEKLGEGQFGEVHLCEVDSPQDLVSLDFPLNVRKGHPLLVAVKILRPDATKNASFSLFSRNDFLKEVKIMSRLKDPNIIRLLGVCVQDDPLCMITDYMENGDLNQFLSAHQLEDKAAEGAPGDGQAAQGPTISYPMLLHVAAQIASGMRYLATLNFVHRDLATRNCLVGENFTIKIADFGMSRNLYAGDYYRVQGRAVLPIRWMAWECILMGKFTTASDVWAFGVTLWEVLMLCRAQPFGQLTDEQVIENAGEFFRDQGRQVYLSRPPACPQGLYELMLRCWSRESEQRPPFSQLHRFLAEDALNTV

SEQ ID NO: 83 - protein, 508 aa, Homo sapiens
MGPEALSSLLLLLLVASGDADMKGHFDPAKCRYALGMQDRTIPDSDISASSSWSDSTAARHSRLESSDGDGAWCPAGSVFPKEEEYLQVDLQRLHLVALVGTQGRHAGGLGKEFSRSYRLRYSRDGRRWMGWKDRWGQEVISGNEDPEGVVLKDLGPPMVARLVRFYPRADRVMSVCLRVELYGCLWRDGLLSYTAPVGQTMYLSEAVYLNDSTYDGHTVGGLQYGGLGQLADGVVGLDDFRKSQELRVWPGYDYVGWSNHSFSSGYVEMEFEFDRLRAFQAMQVHCNNMHTLGARLPGGVECRFRRGPAMAWEGEPMRHNLGGNLGDPRARAVSVPLGGRVARFLQCRFLFAGPWLLFSEISFISDVVNNSSPALGGTFPPAPWWPPGPPPTNFSSLELEPRGQQPVAKAEGSPTAILIGCLVAIILLLLLIIALMLWRLHWRRLLSKAERRVLEEELTVHLSVPGDTILINNRPGPREPPPYQEPRPRGNPPHSAPCVPNGSGAPV

SEQ ID NO: 84 - protein, 767 aa, Homo sapiens
MGPEALSSLLLLLLVASGDADMKGHFDPAKCRYALGMQDRTIPDSDISASSSWSDSTAARHSRLESSDGDGAWCPAGSVFPKEEEYLQVDLQRLHLVALVGTQGRHAGGLGKEFSRSYRLRYSRDGRRWMGWKDRWGQEVISGNEDPEGVVLKDLGPPMVARLVRFYPRADRVMSVCLRVELYGCLWRDGLLSYTAPVGQTMYLSEAVYLNDSTYDGHTVGGLQYGGLGQLADGVVGLDDFRKSQELRVWPGYDYVGWSNHSFSSGYVEMEFEFDRLRAFQAMQVHCNNMHTLGARLPGGVECRFRRGPAMAWEGEPMRHNLGGNLGDPRARAVSVPLGGRVARFLQCRFLFAGPWLLFSEISFISDVVNNSSPALGGTFPPAPWWPPGPPPTNFSSLELEPRGQQPVAKAEGSPTAILIGCLVAIILLLLLIIALMLWRLHWRRLLSKVLESHPRTRSPGLVGIRPTPLPVSPMALVHLCEVDSPQDLVSLDFPLNVRKGHPLLVAVKILRPDATKNARNDFLKEVKIMSRLKDPNIIRLLGVCVQDDPLCMITDYMENGDLNQFLSAHQLEDKAAEGAPGDGQAAQGPTISYPMLLHVAAQIASGMRYLATLNFVHRDLATRNCLVGENFTIKIADFGMSRNLYAGDYYRVQGRAVLPIRWMAWECILMGKFTTASDVWAFGVTLWEVLMLCRAQPFGQLTDEQVIENAGEFFRDQGRQVYLSRPPACPQGLYELMLRCWSRESEQRPPFSQLHRFLAEDALNTV

SEQ ID NO: 85 - protein, 452 aa, Artificial Sequence
  an artificially synthesized sequence
QSVEESGGRLVTPGTPLTLTCTVSGFSLSTSAMSWVRQAPGKGLEWIGMITYGGSGSTWYASWANGRFTISKTSTTVTLKMTSPTTEDTASYFCARVYGTIGSNFYSIYSFNLWGQGTLVTVSSASTKGPSVFPLAPSSKSTSGGTAALGCLVKDYFPEPVTVSWNSGALTSGVHTFPAVLQSSGLYSLSSVVTVPSSSLGTQTYICNVNHKPSNTKVDKRVEPKSCDKTHTCPPCPAPELRRGPSVFLFPPKPKDTLMISRTPEVTCVVVDVSHEDPEVKFNWYVDGVEVHNAKTKPREEQYNSTYRVVSVLTVLHQDWLNGKEYKCKVSNKALPAPIEKTISKAKGQPREPQVYTLPPSREEMTKNQVSLTCLVKGFYPSDIAVEWESNGQPENNYKTTPPVLDSDGSFFLYSKLTVDKSRWQQGNVFSCSVMHEALHNHYTQKSLSLSP

SEQ ID NO: 86 - protein, 218 aa, Artificial Sequence
  an artificially synthesized sequence
AAVLTQTPSPVSAAVGGTVSISCQSSKSVYNSNYLSWYQQKPGQPPKLLIYYTSALASGVSSRFKGSGSGTRFTLTISDVQCDDAATYYCAGGYSSSSDNGFGGGTKVEIKRTVAAPSVFIFPPSDEQLKSGTASVVCLLNNFYPREAKVQWKVDNALQSGNSQESVTEQDSKDCTYSLSSTLTLSKADYEKHKVYACEVTHQGLSSPVTKSFNRGEC

SEQ ID NO: 87 - protein, 444 aa, Artificial Sequence
  an artificially synthesized sequence
QSVEESGGRLITPGTPLTLTCTASGFSLSIYYMIWVRQAPGKGLEWIGYIWSGSTTDYASWAKGRFTISKTSTTVDLKITSPTTEDTATYFCARVYAGYGYGSDLWGQGTLVTVSSASTKGPSVFPLAPSSKSTSGGTAALGCLVKDYFPEPVTVSWNSGALTSGVHTFPAVLQSSGLYSLSSVVTVPSSSLGTQTYICNVNHKPSNTKVDKRVEPKSCDKTHTCPPCPAPELRRGPSVFLFPPKPKDTLMISRTPEVTCVVVDVSHEDPEVKFNWYVDGVEVHNAKTKPREEQYNSTYRVVSVLTVLHQDWLNGKEYKCKVSNKALPAPIEKTISKAKGQPREPQVYTLPPSREEMTKNQVSLTCLVKGFYPSDIAVEWESNGQPENNYKTTPPVLDSDGSFFLYSKLTVDKSRWQQGNVFSCSVMHEALHNHYTQKSLSLSP

SEQ ID NO: 88 - protein, 219 aa, Artificial Sequence
  an artificially synthesized sequence
AAVLTQTPSPVSAAVGGTVSISCQSSQSVYNNNWLAWYQQKPGQPPKLLIYSASTLASGVPSRFKGSGSGTQFTLTISDVQCDDAATYYCAGGYSTNSDKNAFGGGTKVEIKRTVAAPSVFIFPPSDEQLKSGTASVVCLLNNFYPREAKVQWKVDNALQSGNSQESVTEQDSKDCTYSLSSTLTLSKADYEKHKVYACEVTHQGLSSPVTKSFNRGEC

SEQ ID NO: 89 - protein, 440 aa, Artificial Sequence
  an artificially synthesized sequence
QSVEESGGRLVTPGTALTLTCTASGFSLSSYDMSWVRQAPGEGLEWIGTIFTEGSTSCASWVKGRFTISRTSTTVDLKITSPTTEDTATYFCVRGTTSNRLWGQGTLVTVSSASTKGPSVFPLAPSSKSTSGGTAALGCLVKDYFPEPVTVSWNSGALTSGVHTFPAVLQSSGLYSLSSVVTVPSSSLGTQTYICNVNHKPSNTKVDKRVEPKSCDKTHTCPPCPAPELRRGPSVFLFPPKPKDTLMISRTPEVTCVVVDVSHEDPEVKFNWYVDGVEVHNAKTKPREEQYNSTYRVVSVLTVLHQDWLNGKEYKCKVSNKALPAPIEKTISKAKGQPREPQVYTLPPSREEMTKNQVSLTCLVKGFYPSDIAVEWESNGQPENNYKTTPPVLDSDGSFFLYSKLTVDKSRWQQGNVFSCSVMHEALHNHYTQKSLSLSP

SEQ ID NO: 90 - protein, 219 aa, Artificial Sequence
  an artificially synthesized sequence
DVVMTQTPASVEAVVGATVTIRCQASESITNYLSWYQQKPGQPPKVLIYYASTLESGVPSRFKGSGSGTQFTLTISDLECADAATYYCQSNYFSSSYSYGNTFGGGTKVEIKRTVAAPSVFIFPPSDEQLKSGTASVVCLLNNFYPREAKVQWKVDNALQSGNSQESVTEQDSKDCTYSLSSTLTLSKADYEKHKVYACEVTHQGLSSPVTKSFNRGEC

SEQ ID NO: 91 - protein, 449 aa, Artificial Sequence
  an artificially synthesized sequence
QSVEESGGRLVTPGTPLTLTCTVSGFSLSSYSMGWVRQAPGKGLEYIGVINTSDSAYYASWAKGRFTISRTSTTVDLKMTSLTTEDTATYFCARAIGYYGSGWGACYFNLWGQGTLVTVSSASTKGPSVFPLAPSSKSTSGGTAALGCLVKDYFPEPVTVSWNSGALTSGVHTFPAVLQSSGLYSLSSVVTVPSSSLGTQTYICNVNHKPSNTKVDKRVEPKSCDKTHTCPPCPAPELRRGPSVFLFPPKPKDTLMISRTPEVTCVVVDVSHEDPEVKFNWYVDGVEVHNAKTKPREEQYNSTYRVVSVLTVLHQDWLNGKEYKCKVSNKALPAPIEKTISKAKGQPREPQVYTLPPSREEMTKNQVSLTCLVKGFYPSDIAVEWESNGQPENNYKTTPPVLDSDGSFFLYSKLTVDKSRWQQGNVFSCSVMHEALHNHYTQKSLSLSP

SEQ ID NO: 92 - protein, 219 aa, Artificial Sequence
  an artificially synthesized sequence
AIKMTQTPSSVSAAVGGTVTVNCQASEDIKSYLAWYQQKPGQPPKLLIYSASTLASGVSSRFKGSGSGTQFTLTISDLECADAATYYCQSYYGTSTTGEYNAFGGGTKVEIKRTVAAPSVFIFPPSDEQLKSGTASVVCLLNNFYPREAKVQWKVDNALQSGNSQESVTEQDSKDCTYSLSSTLTLSKADYEKHKVYACEVTHQGLSSPVTKSFNRGEC

SEQ ID NO: 93 - protein, 443 aa, Artificial Sequence
  an artificially synthesized sequence
QSLEESGGRLVTPGTPLTLTCTASGFSLSNYYMQWVRQAPGKGLEWIGIVYPGSSAYYANWAKGRFTISKTSTTVDLKMTSLTTEDTATYFCAGSSNSVYSFNLWGQGTLVTVSSASTKGPSVFPLAPSSKSTSGGTAALGCLVKDYFPEPVTVSWNSGALTSGVHTFPAVLQSSGLYSLSSVVTVPSSSLGTQTYICNVNHKPSNTKVDKRVEPKSCDKTHTCPPCPAPELRRGPSVFLFPPKPKDTLMISRTPEVTCVVVDVSHEDPEVKFNWYVDGVEVHNAKTKPREEQYNSTYRVVSVLTVLHQDWLNGKEYKCKVSNKALPAPIEKTISKAKGQPREPQVYTLPPSREEMTKNQVSLTCLVKGFYPSDIAVEWESNGQPENNYKTTPPVLDSDGSFFLYSKLTVDKSRWQQGNVFSCSVMHEALHNHYTQKSLSLSP

SEQ ID NO: 94 - protein, 217 aa, Artificial Sequence
  an artificially synthesized sequence
AYDMTQTPSSVSAAVGGTVTIKCQASESIYRSLAWYQQKPGQPPKLLIYSASTLTSGVSSRFKGSGSGTEFTLTISDLECADAGTYYCQQGGSFSNIVNTFGGGTKVEIKRTVAAPSVFIFPPSDEQLKSGTASVVCLLNNFYPREAKVQWKVDNALQSGNSQESVTEQDSKDCTYSLSSTLTLSKADYEKHKVYACEVTHQGLSSPVTKSFNRGEC

SEQ ID NO: 95 - protein, 441 aa, Artificial Sequence
  an artificially synthesized sequence
QSVEESGGRLVTPGTPLTLTCTVSGFSLSSYSVAWVRQAPGKGLEWIGYISYSGSTYYASWVNGRFTISKTSTTVDLKMTSLTASDTATYFCARDPGYSRDLWGQGTLVTVSSASTKGPSVFPLAPSSKSTSGGTAALGCLVKDYFPEPVTVSWNSGALTSGVHTFPAVLQSSGLYSLSSVVTVPSSSLGTQTYICNVNHKPSNTKVDKRVEPKSCDKTHTCPPCPAPELRRGPSVFLFPPKPKDTLMISRTPEVTCVVVDVSHEDPEVKFNWYVDGVEVHNAKTKPREEQYNSTYRVVSVLTVLHQDWLNGKEYKCKVSNKALPAPIEKTISKAKGQPREPQVYTLPPSREEMTKNQVSLTCLVKGFYPSDIAVEWESNGQPENNYKTTPPVLDSDGSFFLYSKLTVDKSRWQQGNVFSCSVMHEALHNHYTQKSLSLSP

SEQ ID NO: 96 - protein, 216 aa, Artificial Sequence
  an artificially synthesized sequence
DVVMTQTPSSVSEPVGGTVTIKCQASQSIGSYLSWYQQKPGQPPKLLIYRASTLASGVSSRFKGSGSGTEFTLTINGLECADAAIYYCQSSYVGVSHGSFGGGTKVEIKRTVAAPSVFIFPPSDEQLKSGTASVVCLLNNFYPREAKVQWKVDNALQSGNSQESVTEQDSKDCTYSLSSTLTLSKADYEKHKVYACEVTHQGLSSPVTKSFNRGEC

SEQ ID NO: 97 - protein, 443 aa, Artificial Sequence
  an artificially synthesized sequence
QSLEESGGRLVTPGGSLTLTCTASGFSLSAYYMQWVRQAPGKGLEWIGWINTGGSAYYPSWARGRFTISKTSTTVDLKITSPTTEDTATYFCARSDASVHQFNLWGQGTLVTVSSASTKGPSVFPLAPSSKSTSGGTAALGCLVKDYFPEPVTVSWNSGALTSGVHTFPAVLQSSGLYSLSSVVTVPSSSLGTQTYICNVNHKPSNTKVDKRVEPKSCDKTHTCPPCPAPELRRGPSVFLFPPKPKDTLMISRTPEVTCVVVDVSHEDPEVKFNWYVDGVEVHNAKTKPREEQYNSTYRVVSVLTVLHQDWLNGKEYKCKVSNKALPAPIEKTISKAKGQPREPQVYTLPPSREEMTKNQVSLTCLVKGFYPSDIAVEWESNGQPENNYKTTPPVLDSDGSFFLYSKLTVDKSRWQQGNVFSCSVMHEALHNHYTQKSLSLSP

SEQ ID NO: 98 - protein, 218 aa, Artificial Sequence
  an artificially synthesized sequence
DVVMTQTPASVEAAVGGTVTIKCQASESIGNALAWYQQRPGQPPKLLIYYASTLESGVPSRFKGSGSGTEFTLTISDLECADAATYYCQCTYGSGSSRGNAFGGGTKVEIKRTVAAPSVFIFPPSDEQLKSGTASVVCLLNNFYPREAKVQWKVDNALQSGNSQESVTEQDSKDCTYSLSSTLTLSKADYEKHKVYACEVTHQGLSSPVTKSFNRGEC

SEQ ID NO: 99 - protein, 442 aa, Artificial Sequence
  an artificially synthesized sequence
QSVEESGGRLVTPGTPLTLTCAVSGFSLNSHVMGWVRQAPGRGLECIGIIAVSGDIYYANWAKGRFTISKTSTTVDLRITSPTTEDTATYFCGSPTVINNNNLWGQGTLVTVSSASTKGPSVFPLAPSSKSTSGGTAALGCLVKDYFPEPVTVSWNSGALTSGVHTFPAVLQSSGLYSLSSVVTVPSSSLGTQTYICNVNHKPSNTKVDKRVEPKSCDKTHTCPPCPAPELRRGPSVFLFPPKPKDTLMISRTPEVTCVVVDVSHEDPEVKFNWYVDGVEVHNAKTKPREEQYNSTYRVVSVLTVLHQDWLNGKEYKCKVSNKALPAPIEKTISKAKGQPREPQVYTLPPSREEMTKNQVSLTCLVKGFYPSDIAVEWESNGQPENNYKTTPPVLDSDGSFFLYSKLTVDKSRWQQGNVFSCSVMHEALHNHYTQKSLSLSP

SEQ ID NO: 100 - protein, 220 aa, Artificial Sequence
  an artificially synthesized sequence
AQVLTQTASPVSAAVGGTVTINCQSSQNVYGNNYLSWFQQKPGQPPKLLIYSTSTLASGVSSRFKGSGSGTQFTLTISDLECADAATYYCLGGYDCNIVDCRAFGGGTKVEIKRTVAAPSVFIFPPSDEQLKSGTASVVCLLNNFYPREAKVQWKVDNALQSGNSQESVTEQDSKDCTYSLSSTLTLSKADYEKHKVYACEVTHQGLSSPVTKSFNRGEC

SEQ ID NO: 101 - protein, 444 aa, Artificial Sequence
  an artificially synthesized sequence
QSVEESGGRLVTPGTPLTLTCTVSGFSLNRYTGIWVRQAPGKGLEWIGIISSDDRTWYASWAKGRFTISKTSTTVDLKITSPTIEDTATYFCARDVGGDSWFWGLWGQGTLVTVSSASTKGPSVFPLAPSSKSTSGGTAALGCLVKDYFPEPVTVSWNSGALTSGVHTFPAVLQSSGLYSLSSVVTVPSSSLGTQTYICNVNHKPSNTKVDKRVEPKSCDKTHTCPPCPAPELRRGPSVFLFPPKPKDTLMISRTPEVTCVVVDVSHEDPEVKFNWYVDGVEVHNAKTKPREEQYNSTYRVVSVLTVLHQDWLNGKEYKCKVSNKALPAPIEKTISKAKGQPREPQVYTLPPSREEMTKNQVSLTCLVKGFYPSDIAVEWESNGQPENNYKTTPPVLDSDGSFFLYSKLTVDKSRWQQGNVFSCSVMHEALHNHYTQKSLSLSP

SEQ ID NO: 102 - protein, 220 aa, Artificial Sequence
  an artificially synthesized sequence
DIVMTQTPASVEAAVGGTVTIKCQASQSISSWLAWYQQKPGQPPKLLIYYASTLASGVPSRFSGSGSGTEFTLTISDLECADAATYYCQSNYYSSSNSNYGHAFGGGTKVEIKRTVAAPSVFIFPPSDEQLKSGTASVVCLLNNFYPREAKVQWKVDNALQSGNSQESVTEQDSKDCTYSLSSTLTLSKADYEKHKVYACEVTHQGLSSPVTKSFNRGEC